European Patent Specification EP 3 353 194 B1, published August 30, 2023. Title: OMPG VARIANTS. Applicant: GENIA TECHNOLOGIES, INC. The sequence listing filed with the application follows.

SEQUENCE LISTING (23 sequences)

SEQ ID NO: 1 - protein, 301 aa, Escherichia coli
MKKLLPCTALVMCAGMACAQAEERNDWHFNIGAMYEIENVEGYGEDMDGLAEPSVYFNAANGPWRIALAYYQEGPVDYSAGKRGTWFDRPELEVHYQFLENDDFSFGLTGGFRNYGYHYVDEPGKDTANMQRWKIAPDWDVKLTDDLRFNGWLSMYKFANDLNTTGYADTRVETETGLQYTFNETVALRVNYYLERGFNMDDSRNNGEFSTQEIRAYLPLTLGNHSVTPYTRIGLDRWSNWDWQDDIEREGHDFNRVGLFYGYDFQNGLSVSLEYAFEWQDHDEGDSDKFHYAGVGVNYSF

SEQ ID NO: 2 - protein, 280 aa, Escherichia coli
EERNDWHFNIGAMYEIENVEGYGEDMDGLAEPSVYFNAANGPWRIALAYYQEGPVDYSAGKRGTWFDRPELEVHYQFLENDDFSFGLTGGFRNYGYHYVDEPGKDTANMQRWKIAPDWDVKLTDDLRFNGWLSMYKFANDLNTTGYADTRVETETGLQYTFNETVALRVNYYLERGFNMDDSRNNGEFSTQEIRAYLPLTLGNHSVTPYTRIGLDRWSNWDWQDDIEREGHDFNRVGLFYGYDFQNGLSVSLEYAFEWQDHDEGDSDKFHYAGVGVNYSF

SEQ ID NO: 3 - protein, 299 aa, Artificial Sequence
  source: /note="Description of Artificial Sequence: Synthetic polypeptide"
EERNDWHFNIGAMYEIENVEGYGEDMDGLAEPSVYFNAANGPWRIALAYYQEGPVDYSAGKRGTWFDRPELEVHYQFLENDDFSFGLTGGFRNYGYHYVDEPGKDTANMQRWKIAPDWDVKLTDDLRFNGWLSMYKFANDLNTTGYADTRVETETGLQYTFNETVALRVNYYLERGFNMDDSRNNGEFSTQEIRAYLPLTLGNHSVTPYTRIGLDRAGHDFNRVGLFYGYDFQNGLSVSLEYAFEWQDHDEGDSDKFHYAGVGVNYSFEKEKEKGSHHHHHHGSGGAHIVMVDAYKPTK

SEQ ID NO: 4 - DNA, 910 bp, Escherichia coli
atgaaaaagttattaccctgtaccgcactggtgatgtgtgcgggaatggcctgcgcacaggccgaggaaaggaacgactggcactttaatatcggcgcgatgtacgaaatagaaaacgtcgagggttatggcgaagatatggatgggctggcggagccttcagtctattttaatgccgccaacgggccgtggagaattgctctggcctattatcaggaagggccggtagattatagcgcgggtaaacgtggaacgtggtttgatcgcccggagctggaggtgcattatcagttcctcgaaaacgatgatttcagtttcggcctgaccggcggtttccgtaattatggttatcactacgttgatgaaccgggtaaagacacggcgaatatgcagcgctggaaaatcgcgccagactgggatgtgaaactgactgacgatttacgtttcaacggttggttgtcgatgtataaatttgccaacgatctgaacactaccggttacgctgatacccgtgtcgaaacggaaacaggtctgcaatataccttcaacgaaacggttgccttgcgagtgaactattatctcgagcgcggcttcaatatggacgacagccgcaataacggtgagttttccacgcaagaaattcgcgcctatttgccgctgacgctcggcaaccactcggtgacgccgtatacgcgcattgggctggatcgctggagtaactgggactggcaggatgatattgaacgtgaaggccatgattttaaccgtgtaggtttattttacggttatgatttccagaacggactttccgtttcgctggaatacgcgtttgagtggcaggatcacgacgaaggcgacagtgataaattccattatgcaggtgtcggcgtaaattactcgttctgataat

SEQ ID NO: 5 - protein, 299 aa, Artificial Sequence; identical to SEQ ID NO: 3
  source: /note="Description of Artificial Sequence: Synthetic polypeptide"

SEQ ID NO: 6 - protein, 299 aa, Artificial Sequence
  source: /note="Description of Artificial Sequence: Synthetic polypeptide"
EERNDWHFNIGAMYEIENVEGYGEDMDGLAEPSVYFNAANGPWRIALAYKQEGPVDYSAGKRGTWFDRPELEVHYQFLENDDFSFGLTGGFRNYGYHYVDEPGKDTANMQRWKIAPDWDVKLTDDLRFNGWLSMYKFANDLNTTGYADTRVETETGLQYTFNETVALRVNYYLERGFNMDDSRNNGEFSTQEIRAYLPLTLGNHSVTPYTRIGLDRAGHDFNRVGLFYGYDFQNGLSVSLEYAFEWQDHDEGDSDKFHYAGVGVNYSFEKEKEKGSHHHHHHGSGGAHIVMVDAYKPTK

SEQ ID NO: 7 - protein, 299 aa, Artificial Sequence
  source: /note="Description of Artificial Sequence: Synthetic polypeptide"
EERNDWHFNIGAMYEIENVEGYGEDMDGLAEPSVYFNAANGPWRIALAYYQEGPVDYSAGKRGTWFDNPELEVHYQFLENDDFSFGLTGGFRNYGYHYVDEPGKDTANMQRWKIAPDWDVKLTDDLRFNGWLSMYKFANDLNTTGYADTRVETETGLQYTFNETVALRVNYYLERGFNMDDSRNNGEFSTQEIRAYLPLTLGNHSVTPYTRIGLDRAGHDFNRVGLFYGYDFQNGLSVSLEYAFEWQDHDEGDSDKFHYAGVGVNYSFEKEKEKGSHHHHHHGSGGAHIVMVDAYKPTK

SEQ ID NO: 8 - protein, 299 aa, Artificial Sequence
  source: /note="Description of Artificial Sequence: Synthetic polypeptide"
EERNDWHFNIGAMYEIENVEGYGEDMDGLAEPSVYFNAANGPWRIALAYYQEGPVDYSAGKRGTWFDRPELEVHYQFLENDDFSFGLTGGFRNYGYHYVDEPGKDTANMQRWKIAPDWDVKLTDDLRFNGWLSMYKFANDLNTTGYADTRVETETGLQYTFNETVALRVNYYLERGFNMDDSRNNGEFSTQEIRAYLPLTLGNHSVTPYTNIGLDRAGHDFNRVGLFYGYDFQNGLSVSLEYAFEWQDHDEGDSDKFHYAGVGVNYSFEKEKEKGSHHHHHHGSGGAHIVMVDAYKPTK

SEQ ID NO: 9 - protein, 299 aa, Artificial Sequence
  source: /note="Description of Artificial Sequence: Synthetic polypeptide"
EERNDWHFNIGAMYEIKNVEGYGEDMDGLAEPSVYFNAANGPWRIALAYYQEGPVDYSAGKRGTWFDRPELEVHYQFLENDDFSFGLTGGFRNYGYHYVDEPGKDTANMQRWKIAPDWDVKLTDDLRFNGWLSMYKFANDLNTTGYADTRVETETGLQYTFNETVALRVNYYLERGFNMDDSRNNGEFSTQEIRAYLPLTLGNHSVTPYTRIGLDRAGHDFNRVGLFYGYDFQNGLSVSLEYAFEWQDHDEGDSDKFHYAGVGVNYSFEKEKEKGSHHHHHHGSGGAHIVMVDAYKPTK

SEQ ID NO: 10 - protein, 298 aa, Artificial Sequence
  source: /note="Description of Artificial Sequence: Synthetic polypeptide"
EERNDWHFNIGAMYEIENVEGYGEDMDGLAEPSVYFNAANGPWRIALAYYQEGPVDYSAGKRGTWFDRPELEVHYQFLENDDFSFGLTGGFRNYGYHYVDEPGKDTANMQRWKIAPDWDVKLTDDLRFNGWLSMYKFANDLNTTGYADTRVETETGLQYTFNETVALRVNYYLERGFNMDDSRNNGEFSTQEIRAYLPLTLGNHSVTPYTRIGLRAGHDFNRVGLFYGYDFQNGLSVSLEYAFEWQDHDEGDSDKFHYAGVGVNYSFEKEKEKGSHHHHHHGSGGAHIVMVDAYKPTK

SEQ ID NO: 11 - protein, 298 aa, Artificial Sequence
  source: /note="Description of Artificial Sequence: Synthetic polypeptide"
EERNDWHFNIGAMYEIENVEGYGEDMDGLAEPSVYFNAANGPWRIALAYKQEGPVDYSAGKRGTWFDRPELEVHYQFLENDDFSFGLTGGFRNYGYHYVDEPGKDTANMQRWKIAPDWDVKLTDDLRFNGWLSMYKFANDLNTTGYADTRVETETGLQYTFNETVALRVNYYLERGFNMDDSRNNGEFSTQEIRAYLPLTLGNHSVTPYTRIGLRAGHDFNRVGLFYGYDFQNGLSVSLEYAFEWQDHDEGDSDKFHYAGVGVNYSFEKEKEKGSHHHHHHGSGGAHIVMVDAYKPTK

SEQ ID NO: 12 - protein, 301 aa, Shigella flexneri
MKKLLPCTALVMCAGMACAQAEEKNDWHFNIGAMYEIENVEGYGEDMDGLAEPSVYFNAANGPWRIALAYYQEGPVDYSAGKRGTWFDRPELEVHYQFLESDDFSFGLTGGFRNYGYHYVDEPGKDTANMQRWKIAPDWDVKLTDDLRFNGWLSMYKFANDLNTTGYADTRVETETGLQYTFNETVALRVNYYLERGFNMDDSRNNGEFSTQEIRAYLPLTLGNHSVTPYTRIGLDRWSNWDWQDDIEREGHDFNRVGLFYGYDFQNGLSVSLEYAFEWQDHDEGDSDKFHYAGVGVNYSF

SEQ ID NO: 13 - protein, 301 aa, Salmonella enterica
MKTLLSSTALVMCAGMACAQAAEKNDWHFNIGAMYEIENVEGQAEDMDGLGEPSIYFNAANGPWKISLAYYQEGPVDYSAGKRGTWFDRPELEIRYQLLESDDVNFGLTGGFRNYGYHYVDEPGKDTANMQRWKVQPDWDIKLSDDLRFGGWLAMYQFVNELSITGYSDSRVESETGFTYKINDMFSMVTNYYLERGFNIDKSRNNGEFSTQEIRAYLPISLGNTTLTPYTRIGLDRWTNWDWQDDPEREGHDFNRLGLLYAYDFQNGLSMTLEYAFECEDHDEGESDKFHYAGIGINYAF

SEQ ID NO: 14 - protein, 301 aa, Salmonella enterica
MKTLLSSTALVMCAGMACAQAAEKNDWHFNVGAMYEIENVEGQGENMDGLAEPSIYFNAANGPWRISVAYYQEGPVDYSAGKRGTWFDRPEFEVHYQFLESDDVNFGLTGGFRNYGYHYVDEPGKDTANMQRWKVQPDWDIKLSDDLRFGGWFAMYQFVNDLSITGYSDSRVETETGFTYKINDTFSMVTNYYLERGFNIDKSRNNGEFSTQEIRAYLPISLGNTTLTPYTRLGLDRWSNWDWQDDPEREGHDFNRLGLLYAYDFQNGLSMTLEYAFEWEDHDEGESDKFHYAGVGINYAF

SEQ ID NO: 15 - protein, 301 aa, Citrobacter farmeri
MKTLLSTTALMLCAAISCAQAAEKNDWHFNIGAMYEIENVEGYGEDMDGLAEPSVYFNAANGPWRISLAYYQEGPVDYSAGKRGTWFDRPELEVHYQIQESDEFSFGLTGGFRNYGYHYVNEAGKDTANMQRWKVQPDWDVKITDDLRFSGWLSMYQFVNDLSTTGYADSRLESETGLHYTFNETVGVIVNYYLERGFNLADHRNNGEFSTQEIRAYLPLSLGNTTLTPYTRIGLDRWSNWDWRDDPEREGHDFNRLGLQYAYDFQNGLSMTLEYAYEWEDHDEGESDRFHYAGVGVNYAF

SEQ ID NO: 16 - protein, 31 aa, Artificial Sequence
  source: /note="Description of Artificial Sequence: Synthetic polypeptide"
EKEKEKGSHHHHHHGSGGAHIVMVDAYKPTK

SEQ ID NO: 17 - protein, 302 aa, Artificial Sequence
  source: /note="Description of Artificial Sequence: Synthetic polypeptide"
MDKFHYAGVGVNYSFGSGEERNDWHFNIGAMYEIENVEGYGEDMDGLAEPSVYFNAANGPWRIALAYKQEGPVDYSAGKRGTWFDRPELEVHYQFLENDDFSFGLTGGFRNYGYHYVDEPGKDTANMQRWKIAPDWDVKLTDDLRFNGWLSMYKFANDLNTTGYADTRVETETGLQYTFNETVALRVNYYLERGFNMDDSRNNGEFSTQEIRAYLPLTLGNHSVTPYTRIGLRAGHDFNRVGLFYGYDFQNGLSVSLEYAFEWQDHDEGDSEKEKEKGSHHHHHHGSGGAHIVMVDAYKPTK

SEQ ID NO: 18 - protein, 6 aa, Artificial Sequence
  source: /note="Description of Artificial Sequence: Synthetic 6xHis tag"
HHHHHH

SEQ ID NO: 19 - protein, 15 aa, Artificial Sequence
  source: /note="Description of Artificial Sequence: Synthetic peptide"
GGGGSGGGGSGGGGS

SEQ ID NO: 20 - protein, 8 aa, Artificial Sequence
  source: /note="Description of Artificial Sequence: Synthetic peptide"
EKEKEKGS

SEQ ID NO: 21 - protein, 11 aa, Artificial Sequence
  source: /note="Description of Artificial Sequence: Synthetic peptide"
HHHHHHGSGGK

SEQ ID NO: 22 - protein, 13 aa, Artificial Sequence
  source: /note="Description of Artificial Sequence: Synthetic peptide"
AHIVMVDAYKPTK

SEQ ID NO: 23 - protein, 5 aa, Artificial Sequence
  source: /note="Description of Artificial Sequence: Synthetic peptide"
RSKLG